European Patent Application EP 4 467 567 A1, published November 27, 2024. Title: ANTI-CD70 NANOANTIBODY AND USE THEREOF. Applicant: HRAIN BIOTECHNOLOGY CO., LTD. The sequence listing filed with the application follows.

SEQUENCE LISTING (52 sequences)

SEQ ID NO: 1 - protein, 8 aa, Artificial Sequence
  CDR1
GSIFSINA

SEQ ID NO: 2 - protein, 8 aa, Artificial Sequence
  CDR1
GSIFSMNA

SEQ ID NO: 3 - protein, 8 aa, Artificial Sequence
  CDR1
RSIFSINA

SEQ ID NO: 4 - protein, 8 aa, Artificial Sequence
  CDR1
GFTLDGYA

SEQ ID NO: 5 - protein, 8 aa, Artificial Sequence
  CDR1
GNIFSNNA

SEQ ID NO: 6 - protein, 8 aa, Artificial Sequence
  CDR1
GRTSSTYA

SEQ ID NO: 7 - protein, 8 aa, Artificial Sequence
  CDR1
GFTLDYYA

SEQ ID NO: 8 - protein, 10 aa, Artificial Sequence
  CDR2
CDRITSGGST

SEQ ID NO: 9 - protein, 8 aa, Artificial Sequence
  CDR2
ISSSDGST

SEQ ID NO: 10 - protein, 7 aa, Artificial Sequence
  CDR2
ITSDGST

SEQ ID NO: 11 - protein, 8 aa, Artificial Sequence
  CDR2
IGWSGGRT

SEQ ID NO: 12 - protein, 8 aa, Artificial Sequence
  CDR2
ITWSGGRT

SEQ ID NO: 13 - protein, 8 aa, Artificial Sequence
  CDR2
ISSSSDGS

SEQ ID NO: 14 - protein, 12 aa, Artificial Sequence
  CDR3
NAGAGRAFPGDY

SEQ ID NO: 15 - protein, 12 aa, Artificial Sequence
  CDR3
NSGAGRAFPGDY

SEQ ID NO: 16 - protein, 16 aa, Artificial Sequence
  CDR3
TTDVLTSCRSDRWLEV

SEQ ID NO: 17 - protein, 12 aa, Artificial Sequence
  CDR3
NAGAGRAFPGDY

SEQ ID NO: 18 - protein, 19 aa, Artificial Sequence
  CDR3
AADSEQSSSSEGQAYGYED

SEQ ID NO: 19 - protein, 18 aa, Artificial Sequence
  CDR3
AADSEVSSSSEGQYGYES

SEQ ID NO: 20 - protein, 17 aa, Artificial Sequence
  CDR3
CSTDVLTSCRSDRYLEV

SEQ ID NO: 21 - protein, 118 aa, Artificial Sequence
  VHH
EVQLVESGGGLVQAGGSLRLSCAASGSIFSINAMGWYRQAPGKQRELVAAITSGGSTNYADSVKGRFTISRDNAKNTVYLQMNSLKPEDTAVYYCNAGAGRAFPGDYWGQGTQVTVSS

SEQ ID NO: 22 - protein, 118 aa, Artificial Sequence
  VHH
QVQLVESGGGLVQAGGSLRLSCAASGSIFSMNAMGWYRQAPGKQRELVAAITSGGSTNYVDSVKGRFTISRDNAKNTVYLQMNSLKPEDTAVYYCNAGAGRAFPGDYWGQGTQVTVSS

SEQ ID NO: 23 - protein, 118 aa, Artificial Sequence
  VHH
EVQVVESGGGLVQPGGSLRLSCAASRSIFSINAMGWYRQAPGKQRELVAAITSGGSTNYADSVKGRFTISRDNAKNTVYLQMNSLKPEDTAVYYCNSGAGRAFPGDYWGQGTLVTVSS

SEQ ID NO: 24 - protein, 123 aa, Artificial Sequence
  VHH
EVQLVESGGGFVQPGGSLRLSCAASGFTLDGYAVAWFRQAPGKEREGVSCISSSDGSTYYIDSVQGRFTITRNNAKNTVYLQMNSLKPEDTAVYYCTTDVLTSCRSDRWLEVWGQGTLVTVSS

SEQ ID NO: 25 - protein, 118 aa, Artificial Sequence
  VHH
QVQLVETGGGLVQAGGSLRLSCAASGNIFSNNAMGWYRQAPGKQRELVAAITSDGSTNYVDSVKGRFTISRDNAKNTVLLQMNSLKPEDTAVYYCNAGAGRAFPGDYWGQGTLVTVSS

SEQ ID NO: 26 - protein, 126 aa, Artificial Sequence
  VHH
QLQLVESGGGLVQAGGSLRLSCAVSGRTSSTYAMAWFRQAPGKEREIVAVIGWSGGRTAYADSVKGRFTIAKDNAKNTVSLQMNSLKPEDTGVYYCAADSEQSSSSEGQAYGYEDWGQGTLVTVSS

SEQ ID NO: 27 - protein, 125 aa, Artificial Sequence
  VHH
QLQLVESGGGLVQPGGSLRLSCAVSGRTSSTYAMAWFRQAPGKEREIVAVITWSGGRTAYADSVKGRFTIAKDSAKNTVYLQMNSLKPEDTAVYYCAADSEVSSSSEGQYGYESWGQGTQVTVSS

SEQ ID NO: 28 - protein, 124 aa, Artificial Sequence
  VHH
QVQLVESGGGLVQPGGSLRLSCAASGFTLDYYAVGWFRQAPGKEREGVSCISSSSDGSTYYVDSVLGRFTISRNNAENTVYLQMNSLKPEDTAVYYCSTDVLTSCRSDRYLEVWGQGTLVTVSG

SEQ ID NO: 29 - protein, 346 aa, Artificial Sequence
  CAR
EVQLVESGGGLVQAGGSLRLSCAASGSIFSINAMGWYRQAPGKQRELVAAITSGGSTNYADSVKGRFTISRDNAKNTVYLQMNSLKPEDTAVYYCNAGAGRAFPGDYWGQGTQVTVSSTTTPAPRPPTPAPTIASQPLSLRPEACRPAAGGAVHTRGLDFACDIYIWAPLAGTCGVLLLSLVITLYCRFSVVKRGRKKLLYIFKQPFMRPVQTTQEEDGCSCRFPEEEEGGCELRVKFSRSADAPAYQQGQNQLYNELNLGRREEYDVLDKRRGRDPEMGGKPRRKNPQEGLYNELQKDKMAEAYSEIGMKGERRRGKGHDGLYQGLSTATKDTYDALHMQALPPR

SEQ ID NO: 30 - protein, 346 aa, Artificial Sequence
  CAR
QVQLVESGGGLVQAGGSLRLSCAASGSIFSMNAMGWYRQAPGKQRELVAAITSGGSTNYVDSVKGRFTISRDNAKNTVYLQMNSLKPEDTAVYYCNAGAGRAFPGDYWGQGTQVTVSSTTTPAPRPPTPAPTIASQPLSLRPEACRPAAGGAVHTRGLDFACDIYIWAPLAGTCGVLLLSLVITLYCRFSVVKRGRKKLLYIFKQPFMRPVQTTQEEDGCSCRFPEEEEGGCELRVKFSRSADAPAYQQGQNQLYNELNLGRREEYDVLDKRRGRDPEMGGKPRRKNPQEGLYNELQKDKMAEAYSEIGMKGERRRGKGHDGLYQGLSTATKDTYDALHMQALPPR

SEQ ID NO: 31 - protein, 346 aa, Artificial Sequence
  CAR
EVQVVESGGGLVQPGGSLRLSCAASRSIFSINAMGWYRQAPGKQRELVAAITSGGSTNYADSVKGRFTISRDNAKNTVYLQMNSLKPEDTAVYYCNSGAGRAFPGDYWGQGTLVTVSSTTTPAPRPPTPAPTIASQPLSLRPEACRPAAGGAVHTRGLDFACDIYIWAPLAGTCGVLLLSLVITLYCRFSVVKRGRKKLLYIFKQPFMRPVQTTQEEDGCSCRFPEEEEGGCELRVKFSRSADAPAYQQGQNQLYNELNLGRREEYDVLDKRRGRDPEMGGKPRRKNPQEGLYNELQKDKMAEAYSEIGMKGERRRGKGHDGLYQGLSTATKDTYDALHMQALPPR

SEQ ID NO: 32 - protein, 351 aa, Artificial Sequence
  CAR
EVQLVESGGGFVQPGGSLRLSCAASGFTLDGYAVAWFRQAPGKEREGVSCISSSDGSTYYIDSVQGRFTITRNNAKNTVYLQMNSLKPEDTAVYYCTTDVLTSCRSDRWLEVWGQGTLVTVSSTTTPAPRPPTPAPTIASQPLSLRPEACRPAAGGAVHTRGLDFACDIYIWAPLAGTCGVLLLSLVITLYCRFSVVKRGRKKLLYIFKQPFMRPVQTTQEEDGCSCRFPEEEEGGCELRVKFSRSADAPAYQQGQNQLYNELNLGRREEYDVLDKRRGRDPEMGGKPRRKNPQEGLYNELQKDKMAEAYSEIGMKGERRRGKGHDGLYQGLSTATKDTYDALHMQALPPR

SEQ ID NO: 33 - protein, 346 aa, Artificial Sequence
  CAR
QVQLVETGGGLVQAGGSLRLSCAASGNIFSNNAMGWYRQAPGKQRELVAAITSDGSTNYVDSVKGRFTISRDNAKNTVLLQMNSLKPEDTAVYYCNAGAGRAFPGDYWGQGTLVTVSSTTTPAPRPPTPAPTIASQPLSLRPEACRPAAGGAVHTRGLDFACDIYIWAPLAGTCGVLLLSLVITLYCRFSVVKRGRKKLLYIFKQPFMRPVQTTQEEDGCSCRFPEEEEGGCELRVKFSRSADAPAYQQGQNQLYNELNLGRREEYDVLDKRRGRDPEMGGKPRRKNPQEGLYNELQKDKMAEAYSEIGMKGERRRGKGHDGLYQGLSTATKDTYDALHMQALPPR

SEQ ID NO: 34 - protein, 354 aa, Artificial Sequence
  CAR
QLQLVESGGGLVQAGGSLRLSCAVSGRTSSTYAMAWFRQAPGKEREIVAVIGWSGGRTAYADSVKGRFTIAKDNAKNTVSLQMNSLKPEDTGVYYCAADSEQSSSSEGQAYGYEDWGQGTLVTVSSTTTPAPRPPTPAPTIASQPLSLRPEACRPAAGGAVHTRGLDFACDIYIWAPLAGTCGVLLLSLVITLYCRFSVVKRGRKKLLYIFKQPFMRPVQTTQEEDGCSCRFPEEEEGGCELRVKFSRSADAPAYQQGQNQLYNELNLGRREEYDVLDKRRGRDPEMGGKPRRKNPQEGLYNELQKDKMAEAYSEIGMKGERRRGKGHDGLYQGLSTATKDTYDALHMQALPPR

SEQ ID NO: 35 - protein, 353 aa, Artificial Sequence
  CAR
QLQLVESGGGLVQPGGSLRLSCAVSGRTSSTYAMAWFRQAPGKEREIVAVITWSGGRTAYADSVKGRFTIAKDSAKNTVYLQMNSLKPEDTAVYYCAADSEVSSSSEGQYGYESWGQGTQVTVSSTTTPAPRPPTPAPTIASQPLSLRPEACRPAAGGAVHTRGLDFACDIYIWAPLAGTCGVLLLSLVITLYCRFSVVKRGRKKLLYIFKQPFMRPVQTTQEEDGCSCRFPEEEEGGCELRVKFSRSADAPAYQQGQNQLYNELNLGRREEYDVLDKRRGRDPEMGGKPRRKNPQEGLYNELQKDKMAEAYSEIGMKGERRRGKGHDGLYQGLSTATKDTYDALHMQALPPR

SEQ ID NO: 36 - protein, 352 aa, Artificial Sequence
  CAR
QVQLVESGGGLVQPGGSLRLSCAASGFTLDYYAVGWFRQAPGKEREGVSCISSSSDGSTYYVDSVLGRFTISRNNAENTVYLQMNSLKPEDTAVYYCSTDVLTSCRSDRYLEVWGQGTLVTVSGTTTPAPRPPTPAPTIASQPLSLRPEACRPAAGGAVHTRGLDFACDIYIWAPLAGTCGVLLLSLVITLYCRFSVVKRGRKKLLYIFKQPFMRPVQTTQEEDGCSCRFPEEEEGGCELRVKFSRSADAPAYQQGQNQLYNELNLGRREEYDVLDKRRGRDPEMGGKPRRKNPQEGLYNELQKDKMAEAYSEIGMKGERRRGKGHDGLYQGLSTATKDTYDALHMQALPPR

SEQ ID NO: 37 - protein, 231 aa, Artificial Sequence
  CH
PKSCDKTHTCPPCPAPELLGGPSVFLFPPKPKDTLMISRTPEVTCVVVDVSHEDPEVKFNWYVDGVEVHNAKTKPREEQYNSTYRVVSVLTVLHQDWLNGKEYKCKVSNKALPAPIEKTISKAKGQPREPQVYTLPPSRDELTKNQVSLTCLVKGFYPSDIAVEWESNGQPENNYKTTPPVLDSDGSFFLYSKLTVDKSRWQQGNVFSCSVMHEALHNHYTQKSLSLSPGK

SEQ ID NO: 38 - protein, 21 aa, Artificial Sequence
  CD8 SP
MALPVTALLLPLALLLHAARP

SEQ ID NO: 39 - protein, 47 aa, Artificial Sequence
  CD8 hinge
TTTPAPRPPTPAPTIASQPLSLRPEACRPAAGGAVHTRGLDFACDIY

SEQ ID NO: 40 - protein, 22 aa, Artificial Sequence
  CD8 TM
IWAPLAGTCGVLLLSLVITLYC

SEQ ID NO: 41 - protein, 111 aa, Artificial Sequence
  CD3zeta cytoplasmic domain
VKFSRSADAPAYQQGQNQLYNELNLGRREEYDVLDKRRGRDPEMGGKPRRKNPQEGLYNELQKDKMAEAYSEIGMKGERRRGKGHDGLYQGLSTATKDTYDALHMQALPPR

SEQ ID NO: 42 - protein, 48 aa, Artificial Sequence
  41BB cytoplasmic domain
RFSVVKRGRKKLLYIFKQPFMRPVQTTQEEDGCSCRFPEEEEGGCELR

SEQ ID NO: 43 - DNA, 1038 bp, Artificial Sequence
  CAR
gaggtgcagctggtggagtctgggggaggcttggtgcaggctggggggtctctgagactctcctgtgcagcctctggaagcatcttcagtatcaatgccatgggctggtaccgccaggctccagggaagcagcgcgagttggtcgcagctattactagtggtggtagcacaaactatgcagactccgtgaagggccgattcaccatctccagagacaacgccaagaacacggtgtatctgcaaatgaacagcctgaaacctgaggacacagccgtctattactgtaatgcaggagcggggcgggcctttcccggggactactggggccaggggacccaggtcaccgtctcctcaactacaactccagcacccagaccccctacacctgctccaactatcgcaagtcagcccctgtcactgcgccctgaagcctgtcgccctgctgccgggggagctgtgcatactcggggactggactttgcctgtgatatctacatctgggcgcccttggccgggacttgtggggtccttctcctgtcactggttatcaccctttactgcaggttcagtgtcgtgaagagaggccggaagaagctgctgtacatcttcaagcagcctttcatgaggcccgtgcagactacccaggaggaagatggatgcagctgtagattccctgaagaggaggaaggaggctgtgagctgagagtgaagttctcccgaagcgcagatgccccagcctatcagcagggacagaatcagctgtacaacgagctgaacctgggaagacgggaggaatacgatgtgctggacaaaaggcggggcagagatcctgagatgggcggcaaaccaagacggaagaacccccaggaaggtctgtataatgagctgcagaaagacaagatggctgaggcctactcagaaatcgggatgaagggcgaaagaaggagaggaaaaggccacgacggactgtaccaggggctgagtacagcaacaaaagacacctatgacgctctgcacatgcaggctctgccaccaaga

SEQ ID NO: 44 - DNA, 1038 bp, Artificial Sequence
  CAR
caggtgcagctcgtggagtctgggggaggcttggtgcaggctggggggtctctgagactctcctgtgcagcctctggaagcatcttcagtatgaatgccatgggctggtaccgccaggctccagggaagcagcgcgagttggtcgcagctattactagtggtggtagcacaaactatgtagactccgtgaagggccgattcaccatctccagagacaacgccaagaacacggtgtatctgcaaatgaacagcctgaaacctgaggacacagccgtctattactgtaatgcaggagcggggcgggcctttcccggggactactggggccaggggacccaggtcaccgtctcctcaactacaactccagcacccagaccccctacacctgctccaactatcgcaagtcagcccctgtcactgcgccctgaagcctgtcgccctgctgccgggggagctgtgcatactcggggactggactttgcctgtgatatctacatctgggcgcccttggccgggacttgtggggtccttctcctgtcactggttatcaccctttactgcaggttcagtgtcgtgaagagaggccggaagaagctgctgtacatcttcaagcagcctttcatgaggcccgtgcagactacccaggaggaagatggatgcagctgtagattccctgaagaggaggaaggaggctgtgagctgagagtgaagttctcccgaagcgcagatgccccagcctatcagcagggacagaatcagctgtacaacgagctgaacctgggaagacgggaggaatacgatgtgctggacaaaaggcggggcagagatcctgagatgggcggcaaaccaagacggaagaacccccaggaaggtctgtataatgagctgcagaaagacaagatggctgaggcctactcagaaatcgggatgaagggcgaaagaaggagaggaaaaggccacgacggactgtaccaggggctgagtacagcaacaaaagacacctatgacgctctgcacatgcaggctctgccaccaaga

SEQ ID NO: 45 - DNA, 1038 bp, Artificial Sequence
  CAR
gaggtgcaggtcgtggagtctgggggaggcttggtgcagcctggggggtctctgagactctcctgtgcagcctctcgaagcatcttcagtatcaatgccatgggctggtaccgccaggctccagggaaacagcgcgagttggtcgcagctattactagtggtggtagcacaaactatgcagactccgtgaagggccgattcaccatctccagagacaacgccaagaacacggtgtatctgcaaatgaacagcctgaaacctgaggacacagccgtctattactgtaattcaggagcggggcgggcctttcccggggactactggggccaggggaccctggtcaccgtctcctcaactacaactccagcacccagaccccctacacctgctccaactatcgcaagtcagcccctgtcactgcgccctgaagcctgtcgccctgctgccgggggagctgtgcatactcggggactggactttgcctgtgatatctacatctgggcgcccttggccgggacttgtggggtccttctcctgtcactggttatcaccctttactgcaggttcagtgtcgtgaagagaggccggaagaagctgctgtacatcttcaagcagcctttcatgaggcccgtgcagactacccaggaggaagatggatgcagctgtagattccctgaagaggaggaaggaggctgtgagctgagagtgaagttctcccgaagcgcagatgccccagcctatcagcagggacagaatcagctgtacaacgagctgaacctgggaagacgggaggaatacgatgtgctggacaaaaggcggggcagagatcctgagatgggcggcaaaccaagacggaagaacccccaggaaggtctgtataatgagctgcagaaagacaagatggctgaggcctactcagaaatcgggatgaagggcgaaagaaggagaggaaaaggccacgacggactgtaccaggggctgagtacagcaacaaaagacacctatgacgctctgcacatgcaggctctgccaccaaga

SEQ ID NO: 46 - DNA, 1053 bp, Artificial Sequence
  CAR
gaggtgcagctcgtggagtctgggggaggctttgtgcagccgggggggtctctgagactctcctgtgcagcctctggattcactttggatggctatgccgtagcctggttccgccaggccccagggaaagagcgcgagggggtctcatgtattagtagtagtgatggtagcacatactatatagactccgtacagggccgattcaccatcacaagaaacaatgccaagaacacggtgtatctgcaaatgaacagcctgaaacctgaggacacggccgtttattactgtacgacagatgtccttacgagctgccggagcgacaggtggctcgaagtttggggccagggcaccctggtcactgtctcctcaactacaactccagcacccagaccccctacacctgctccaactatcgcaagtcagcccctgtcactgcgccctgaagcctgtcgccctgctgccgggggagctgtgcatactcggggactggactttgcctgtgatatctacatctgggcgcccttggccgggacttgtggggtccttctcctgtcactggttatcaccctttactgcaggttcagtgtcgtgaagagaggccggaagaagctgctgtacatcttcaagcagcctttcatgaggcccgtgcagactacccaggaggaagatggatgcagctgtagattccctgaagaggaggaaggaggctgtgagctgagagtgaagttctcccgaagcgcagatgccccagcctatcagcagggacagaatcagctgtacaacgagctgaacctgggaagacgggaggaatacgatgtgctggacaaaaggcggggcagagatcctgagatgggcggcaaaccaagacggaagaacccccaggaaggtctgtataatgagctgcagaaagacaagatggctgaggcctactcagaaatcgggatgaagggcgaaagaaggagaggaaaaggccacgacggactgtaccaggggctgagtacagcaacaaaagacacctatgacgctctgcacatgcaggctctgccaccaaga

SEQ ID NO: 47 - DNA, 1038 bp, Artificial Sequence
  CAR
caagtgcagctggtggagactgggggaggcttggtgcaggctggggggtctctgagactctcctgtgcagcctctggaaacatcttcagtaacaatgccatgggctggtaccgccaggctccagggaagcagcgcgagttggtcgcagctattactagtgatggtagcacaaactatgtagactccgtgaagggccgattcaccatctccagagacaacgccaagaacacggtgcttctgcaaatgaacagcctgaaacctgaggacacagccgtctattactgtaatgcaggagcggggcgggcctttcccggggactactggggccaggggaccctggtcactgtctcctcaactacaactccagcacccagaccccctacacctgctccaactatcgcaagtcagcccctgtcactgcgccctgaagcctgtcgccctgctgccgggggagctgtgcatactcggggactggactttgcctgtgatatctacatctgggcgcccttggccgggacttgtggggtccttctcctgtcactggttatcaccctttactgcaggttcagtgtcgtgaagagaggccggaagaagctgctgtacatcttcaagcagcctttcatgaggcccgtgcagactacccaggaggaagatggatgcagctgtagattccctgaagaggaggaaggaggctgtgagctgagagtgaagttctcccgaagcgcagatgccccagcctatcagcagggacagaatcagctgtacaacgagctgaacctgggaagacgggaggaatacgatgtgctggacaaaaggcggggcagagatcctgagatgggcggcaaaccaagacggaagaacccccaggaaggtctgtataatgagctgcagaaagacaagatggctgaggcctactcagaaatcgggatgaagggcgaaagaaggagaggaaaaggccacgacggactgtaccaggggctgagtacagcaacaaaagacacctatgacgctctgcacatgcaggctctgccaccaaga

SEQ ID NO: 48 - DNA, 1062 bp, Artificial Sequence
  CAR
cagttgcagctcgtggagtctgggggaggattggtgcaggctgggggctctctaagactctcctgtgcagtttctggacgcacctcaagtacttatgccatggcctggttccgccaggctccaggcaaggagcgtgagattgtagcagttattggatggagtggtggtaggacggcctatgcagactccgtgaagggccgattcactatcgccaaagacaacgccaagaacacggtgtctctgcaaatgaacagtctgaaacctgaggacacgggcgtttattactgtgcagcagattctgaacaaagtagctcgtccgaaggccaggcgtatggctatgaggactggggccaggggaccctggtcactgtctcctcaactacaactccagcacccagaccccctacacctgctccaactatcgcaagtcagcccctgtcactgcgccctgaagcctgtcgccctgctgccgggggagctgtgcatactcggggactggactttgcctgtgatatctacatctgggcgcccttggccgggacttgtggggtccttctcctgtcactggttatcaccctttactgcaggttcagtgtcgtgaagagaggccggaagaagctgctgtacatcttcaagcagcctttcatgaggcccgtgcagactacccaggaggaagatggatgcagctgtagattccctgaagaggaggaaggaggctgtgagctgagagtgaagttctcccgaagcgcagatgccccagcctatcagcagggacagaatcagctgtacaacgagctgaacctgggaagacgggaggaatacgatgtgctggacaaaaggcggggcagagatcctgagatgggcggcaaaccaagacggaagaacccccaggaaggtctgtataatgagctgcagaaagacaagatggctgaggcctactcagaaatcgggatgaagggcgaaagaaggagaggaaaaggccacgacggactgtaccaggggctgagtacagcaacaaaagacacctatgacgctctgcacatgcaggctctgccaccaaga

SEQ ID NO: 49 - DNA, 1059 bp, Artificial Sequence
  CAR
cagttgcagctcgtggagtctgggggaggcttggtgcagcctggggggtccctgagactctcctgtgcagtttctggacgcacctcaagtacttatgccatggcctggttccgccaggctccaggcaaggagcgtgagattgtagcagttattacatggagtggtggtaggacggcctatgcagactccgtgaagggccgattcactatcgccaaagacagcgccaagaacacggtgtatctgcaaatgaacagcctgaaacctgaggatacggccgtttattactgtgcagcagattctgaagtaagcagctcgtccgaaggccagtatggctatgagtcctggggccaggggacccaggtcaccgtctcctcaactacaactccagcacccagaccccctacacctgctccaactatcgcaagtcagcccctgtcactgcgccctgaagcctgtcgccctgctgccgggggagctgtgcatactcggggactggactttgcctgtgatatctacatctgggcgcccttggccgggacttgtggggtccttctcctgtcactggttatcaccctttactgcaggttcagtgtcgtgaagagaggccggaagaagctgctgtacatcttcaagcagcctttcatgaggcccgtgcagactacccaggaggaagatggatgcagctgtagattccctgaagaggaggaaggaggctgtgagctgagagtgaagttctcccgaagcgcagatgccccagcctatcagcagggacagaatcagctgtacaacgagctgaacctgggaagacgggaggaatacgatgtgctggacaaaaggcggggcagagatcctgagatgggcggcaaaccaagacggaagaacccccaggaaggtctgtataatgagctgcagaaagacaagatggctgaggcctactcagaaatcgggatgaagggcgaaagaaggagaggaaaaggccacgacggactgtaccaggggctgagtacagcaacaaaagacacctatgacgctctgcacatgcaggctctgccaccaaga

SEQ ID NO: 50 - DNA, 1056 bp, Artificial Sequence
  CAR
caggtgcagctggtggagtctgggggaggcttggtgcagccgggggggtctctgagactctcctgtgcagcctctggattcactttggattattatgccgtaggctggttccgccaggccccagggaaggagcgcgagggggtctcatgtattagtagtagtagtgatggtagcacatactatgtagactccgtgctgggccgattcaccatctccagaaacaatgccgagaacacggtgtatctgcaaatgaacagcctgaaacctgaggacacggccgtttattactgttcgacagatgtccttacgagctgccggagcgacaggtatctcgaagtttggggccagggcaccctggtcactgtctcaggcactacaactccagcacccagaccccctacacctgctccaactatcgcaagtcagcccctgtcactgcgccctgaagcctgtcgccctgctgccgggggagctgtgcatactcggggactggactttgcctgtgatatctacatctgggcgcccttggccgggacttgtggggtccttctcctgtcactggttatcaccctttactgcaggttcagtgtcgtgaagagaggccggaagaagctgctgtacatcttcaagcagcctttcatgaggcccgtgcagactacccaggaggaagatggatgcagctgtagattccctgaagaggaggaaggaggctgtgagctgagagtgaagttctcccgaagcgcagatgccccagcctatcagcagggacagaatcagctgtacaacgagctgaacctgggaagacgggaggaatacgatgtgctggacaaaaggcggggcagagatcctgagatgggcggcaaaccaagacggaagaacccccaggaaggtctgtataatgagctgcagaaagacaagatggctgaggcctactcagaaatcgggatgaagggcgaaagaaggagaggaaaaggccacgacggactgtaccaggggctgagtacagcaacaaaagacacctatgacgctctgcacatgcaggctctgccaccaaga

SEQ ID NO: 51 - protein, 238 aa, Artificial Sequence
  IgG1Fc
ELKTPQPQSQPECRCPKCPAPELLGGPSVFIFPPKPKDVLSISGRPEVTCVVVDVGQEDPEVSFNWYIDGAEVRTANTKPKEEQFNSTYRVVSVLPIRHQDWLTGKEFKCKVNNKALPAPIERTISKAKGQTREPQVYALAPHREELAKDTVSVTCLVKDFYPVDINIEWQRNGQPESEGTYATTPPQLDNDGTYFLYSKLSVGKNTWQRGETFTCVVMHEALPNHYTQKSITQSSGK

SEQ ID NO: 52 - DNA, 1410 bp, Artificial Sequence
  ARGXBBz
gttgtgacccaggagccttccctgacagtgtctccaggagggacggtcacgctcacctgcggcctcaaatctgggtctgtcacttccgataacttccccacttggtaccagcagacaccaggccaggctccccgattgcttatctacaacacaaacacccgtcactctggcgtccccgaccgcttctccggatccatcctgggcaacaaagccgccctcaccatcacgggggcccaggccgacgacgaggccgaatatttctgtgctctgttcataagtaatcctagtgttgagttcggcggagggacccaactgaccgtcctaggtggcagcaccagcggctccggcaagcctggatctggcgagggcagcaccaagggcgaggtgcagctcgtggagtctgggggaggcttggtgcagcctggggggtctctgagactctcctgtgcagcctctggattcaccttcagtgtctactacatgaactgggtccgccaggctccagggaaggggctcgagtgggtctcagatattaataatgaaggtggtactacatactatgcagactccgtgaagggccgattcaccatctccagagacaactctaagaacagcctgtatctgcaaatgaacagcctgcgcgccgaggacacggccgtgtactactgcgcgagagatgccggatatagcaaccatgtacccatctttgattcttggggccagggcactacaactccagcacccagaccccctacacctgctccaactatcgcaagtcagcccctgtcactgcgccctgaagcctgtcgccctgctgccgggggagctgtgcatactcggggactggactttgcctgtgatatctacatctgggcgcccttggccgggacttgtggggtccttctcctgtcactggttatcaccctttactgcaggttcagtgtcgtgaagagaggccggaagaagctgctgtacatcttcaagcagcctttcatgaggcccgtgcagactacccaggaggaagatggatgcagctgtagattccctgaagaggaggaaggaggctgtgagctgagagtgaagttctcccgaagcgcagatgccccagcctatcagcagggacagaatcagctgtacaacgagctgaacctgggaagacgggaggaatacgatgtgctggacaaaaggcggggcagagatcctgagatgggcggcaaaccaagacggaagaacccccaggaaggtctgtataatgagctgcagaaagacaagatggctgaggcctactcagaaatcgggatgaagggcgaaagaaggagaggaaaaggccacgacggactgtaccaggggctgagtacagcaacaaaagacacctatgacgctctgcacatgcaggctctgccaccaaga